European Patent Specification EP 4 021 571 B1, published October 8, 2025. Title: Therapy Guidance and/or Therapy Monitoring for treatment of shock. Applicant: 4TEEN4 Pharmaceuticals GmbH. The sequence listing filed with the application follows.

SEQUENCE LISTING (44 sequences)

SEQ ID NO: 1 - protein, 737 aa, Homo sapiens
MADTQYILPNDIGVSSLDCREAFRLLSPTERLYAYHLSRAAWYGGLAVLLQTSPEAPYIYALLSRLFRAQDPDQLRQHALAEGLTEEEYQAFLVYAAGVYSNMGNYKSFGDTKFVPNLPKEKLERVILGSEAAQQHPEEVRGLWQTCGELMFSLEPRLRHLGLGKEGITTYFSGNCTMEDAKLAQDFLDSQNLSAYNTRLFKEVDGEGKPYYEVRLASVLGSEPSLDSEVTSKLKSYEFRGSPFQVTRGDYAPILQKVVEQLEKAKAYAANSHQGQMLAQYIESFTQGSIEAHKRGSRFWIQDKGPIVESYIGFIESYRDPFGSRGEFEGFVAVVNKAMSAKFERLVASAEQLLKELPWPPTFEKDKFLTPDFTSLDVLTFAGSGIPAGINIPNYDDLRQTEGFKNVSLGNVLAVAYATQREKLTFLEEDDKDLYILWKGPSFDVQVGLHELLGHGSGKLFVQDEKGAFNFDQETVINPETGEQIQSWYRSGETWDSKFSTIASSYEECRAESVGLYLCLHPQVLEIFGFEGADAEDVIYVNWLNMVRAGLLALEFYTPEAFNWRQAHMQARFVILRVLLEAGEGLVTITPTTGSDGRPDARVRLDRSKIRSVGKPALERFLRRLQVLKSTGDVAGGRALYEGYATVTDAPPECFLTLRDTVLLRKESRKLIVQPNTRLEGSDVQLLEYEASAAGLIRSFSERFPEDGPELEEILTQLATADARFWKGPSEAPSGQA

SEQ ID NO: 2 - protein, 21 aa, Homo sapiens
CETVINPETGEQIQSWYRSGE

SEQ ID NO: 3 - protein, 6 aa, Homo sapiens
INPETG

SEQ ID NO: 4 - protein, 116 aa, Mus musculus
QVTLKESGPGILQPSQTLSLTCSFSGFSLSTSGMSVGWIRQPSGKGLEWLAHIWWNDNKSYNPALKSRLTISRDTSNNQVFLKIASVVTADTGTYFCARNYSYDYWGQGTTLTVSS

SEQ ID NO: 5 - protein, 112 aa, Mus musculus
DVVVTQTPLSLSVSLGDPASISCRSSRSLVHSIGSTYLHWYLQKPGQSPKLLIYKVSNRFSGVPDRFSGSGSGTDFTLKISRVEAEDLGVYFCSQSTHVPWTFGGGTKLEIK

SEQ ID NO: 6 - protein, 10 aa, Mus musculus
GFSLSTSGMS

SEQ ID NO: 7 - protein, 7 aa, Mus musculus
IWWNDNK

SEQ ID NO: 8 - protein, 8 aa, Mus musculus
ARNYSYDY

SEQ ID NO: 9 - protein, 11 aa, Mus musculus
RSLVHSIGSTY

SEQ ID NO: 10 - protein, 9 aa, Mus musculus
SQSTHVPWT

SEQ ID NO: 11 - protein, 469 aa, Homo sapiens
MDPKGSLSWRILLFLSLAFELSYGQITLKESGPTLVKPTQTLTLTCTFSGFSLSTSGMSVGWIRQPPGKALEWLAHIWWNDNKSYNPALKSRLTITRDTSKNQVVLTMTNMDPVDTGTYYCARNYSYDYWGQGTLVTVSSASTKGPSVFPLAPSSKSTSGGTAALGCLVKDYFPEPVTVSWNSGALTSGVHTFPAVLQSSGLYSLSSVVTVPSSSLGTQTYICNVNHKPSNTKVDKKVEPKSCDKTHTCPPCPAPELLGGPSVFLFPPKPKDTLMISRTPEVTCVVVDVSHEDPEVKFNWYVDGVEVHNAKTKPREEQYNSTYRVVSVLTVLHQDWLNGKEYKCKVSNKALPAPIEKTISKAKGQPREPQVYTLPPSRDELTKNQVSLTCLVKGFYPSDIAVEWESNGQPENNYKTTPPVLDSDGSFFLYSKLTVDKSRWQQGNVFSCSVMHEALHNHYTQKSLSLSPG

SEQ ID NO: 12 - protein, 239 aa, Homo sapiens
METDTLLLWVLLLWVPGSTGDIVMTQTPLSLSVTPGQPASISCKSSRSLVHSIGSTYLYWYLQKPGQSPQLLIYKVSNRFSGVPDRFSGSGSGTDFTLKISRVEAEDVGVYYCSQSTHVPWTFGGGTKVEIKRTVAAPSVFIFPPSDEQLKSGTASVVCLLNNFYPREAKVQWKVDNALQSGNSQESVTEQDSKDSTYSLSSTLTLSKADYEKHKVYACEVTHQGLSSPVTKSFNRGEC

SEQ ID NO: 13 - protein, 8 aa, Homo sapiens
DRVYIHPF

SEQ ID NO: 14 - protein, 8 aa, Artificial Sequence
  Angiotensin II variant
DRVYVHPF

SEQ ID NO: 15 - protein, 8 aa, Artificial Sequence
  Angiotensin II variant
NRVFIHPF

SEQ ID NO: 16 - protein, 6 aa, Homo sapiens
VYIHPF

SEQ ID NO: 17 - protein, 9 aa, Homo sapiens
NRVYYVHPF

SEQ ID NO: 18 - protein, 8 aa, Artificial Sequence
  Angiotensin II analogue
NRVYIHPI

SEQ ID NO: 19 - protein, 8 aa, Artificial Sequence
  Angiotensin II analogue
NRVYIHPA

SEQ ID NO: 20 - protein, 8 aa, Artificial Sequence
  Angiotensin II analogue
NRVYIHPF

SEQ ID NO: 21 - protein, 7 aa, Homo sapiens
RVYIHPF

SEQ ID NO: 22 - protein, 7 aa, Artificial Sequence
  Angiotensin III analogue
RVYVHPF

SEQ ID NO: 23 - protein, 7 aa, Artificial Sequence
  Angiotensin III analogue
RVFIHPF

SEQ ID NO: 24 - protein, 7 aa, Artificial Sequence
  Angiotensin III analogue
RVYIHPA

SEQ ID NO: 25 - protein, 7 aa, Artificial Sequence
  Angiotensin III analogue
RVYIHPF

SEQ ID NO: 26 - protein, 6 aa, Homo sapiens
VYIHPF

SEQ ID NO: 27 - protein, 6 aa, Artificial Sequence
  Angiotensin IV analogue
VYVHPF

SEQ ID NO: 28 - protein, 6 aa, Artificial Sequence
  Angiotensin IV analogue
VFIHPF

SEQ ID NO: 29 - protein, 6 aa, Artificial Sequence
  Angiotensing IV analogue
VYIHPA

SEQ ID NO: 30 - protein, 6 aa, Artificial Sequence
  Angiotensin IV analogue
VYIHPF

SEQ ID NO: 31 - protein, 164 aa, Homo sapiens
ARLDVASEFRKKWNKWALSRGKRELRMSSSYPTGLADVKAGPAQTLIRPQDMKGASRSPEDSSPDAARIRVKRYRQSMNNFQGLRSFGCRFGTCTVQKLAHQIYQFTDKDKDNVAPRSKISPQGYGRRRRRSLPEAGPGRTLVSSKPQAHGAPAPPSGSAPHFL

SEQ ID NO: 32 - protein, 20 aa, Homo sapiens
ARLDVASEFRKKWNKWALSR

SEQ ID NO: 33 - protein, 48 aa, Homo sapiens
ELRMSSSYPTGLADVKAGPAQTLIRPQDMKGASRSPEDSSPDAARIRV

SEQ ID NO: 34 - protein, 52 aa, Artificial Sequence
  C-terminal amide (CONH2)
YRQSMNNFQGLRSFGCRFGTCTVQKLAHQIYQFTDKDKDNVAPRSKISPQGY

SEQ ID NO: 35 - protein, 53 aa, Artificial Sequence
  Glycine at C-terminus
YRQSMNNFQGLRSFGCRFGTCTVQKLAHQIYQFTDKDKDNVAPRSKISPQGYG

SEQ ID NO: 36 - protein, 38 aa, Homo sapiens
RRRRRSLPEAGPGRTLVSSKPQAHGAPAPPSGSAPHFL

SEQ ID NO: 37 - protein, 21 aa, Homo sapiens
YRQSMNNFQGLRSFGCRFGTC

SEQ ID NO: 38 - protein, 8 aa, Homo sapiens
GYTFSRYW

SEQ ID NO: 39 - protein, 8 aa, Homo sapiens
ILPGSGST

SEQ ID NO: 40 - protein, 11 aa, Homo sapiens
TEGYEYDGFDY

SEQ ID NO: 41 - protein, 11 aa, Homo sapiens
QSIVYSNGNTY

SEQ ID NO: 42 - protein, 9 aa, Homo sapiens
FQGSHIPYT

SEQ ID NO: 43 - protein, 448 aa, Homo sapiens
QVQLVQSGAEVKKPGSSVKVSCKASGYTFSRYWIEWVRQAPGQGLEWIGEILPGSGSTNYNQKFQGRVTITADTSTSTAYMELSSLRSEDTAVYYCTEGYEYDGFDYWGQGTTVTVSSASTKGPSVFPLAPSSKSTSGGTAALGCLVKDYFPEPVTVSWNSGALTSGVHTFPAVLQSSGLYSLSSVVTVPSSSLGTQTYICNVNHKPSNTKVDKKVEPKSCDKTHTCPPCPAPELLGGPSVFLFPPKPKDTLMISRTPEVTCVVVDVSHEDPEVKFNWYVDGVEVHNAKTKPREEQYNSTYRVVSVLTVLHQDWLNGKEYKCKVSNKALPAPIEKTISKAKGQPREPQVYTLPPSRDELTKNQVSLTCLVKGFYPSDIAVEWESNGQPENNYKTTPPVLDSDGSFFLYSKLTVDKSRWQQGNVFSCSVMHEALHNHYTQKSLSLSPGK

SEQ ID NO: 44 - protein, 219 aa, Homo sapiens
DVVLTQSPLSLPVTLGQPASISCRSSQSIVYSNGNTYLEWYLQRPGQSPRLLIYRVSNRFSGVPDRFSGSGSGTDFTLKISRVEAEDVGVYYCFQGSHIPYTFGGGTKLEIKRTVAAPSVFIFPPSDEQLKSGTASVVCLLNNFYPREAKVQWKVDNALQSGNSQESVTEQDSKDSTYSLSSTLTLSKADYEKHKVYACEVTHQGLSSPVTKSFNRGEC